European Patent Application EP 4 273 224 A1, published November 8, 2023. Title: RECOMBINANT MICROORGANISM, PREPARATION METHOD THEREFOR, AND APPLICATION OF RECOMBINANT MICROORGANISM IN PRODUCTION OF TAGATOSE. Applicant: TIANJIN INSTITUTE OF INDUSTRIAL BIOTECHNOLOGY, CHINESE ACADEMY OF SCIENCES. The sequence listing filed with the application follows.

SEQUENCE LISTING (55 sequences)

SEQ ID NO: 1 - protein, 477 aa, Escherichia coli
MFKNAFANLQKVGKSLMLPVSVLPIAGILLGVGSANFSWLPAVVSHVMAEAGGSVFANMPLIFAIGVALGFTNNDGVSALAAVVAYGIMVKTMAVVAPLVLHLPAEEIASKHLADTGVLGGIISGAIAAYMFNRFYRIKLPEYLGFFAGKRFVPIISGLAAIFTGVVLSFIWPPIGSAIQTFSQWAAYQNPVVAFGIYGFIERCLVPFGLHHIWNVPFQMQIGEYTNAAGQVFHGDIPRYMAGDPTAGKLSGGFLFKMYGLPAAAIAIWHSAKPENRAKVGGIMISAALTSFLTGITEPIEFSFMFVAPILYIIHAILAGLAFPICILLGMRDGTSFSHGLIDFIVLSGNSSKLWLFPIVGIGYAIVYYTIFRVLIKALDLKTPGREDATEDAKATGTSEMAPALVAAFGGKENITNLDACITRLRVSVADVSKVDQAGLKKLGAAGVVVAGSGVQAIFGTKSDNLKTEMDEYIRNH

SEQ ID NO: 2 - DNA, 1431 bp, Escherichia coli
atgtttaagaatgcatttgctaacctgcaaaaggtcggtaaatcgctgatgctgccggtatccgtactgcctatcgcaggtattctgctgggcgtcggttccgcgaatttcagctggctgcccgccgttgtatcgcatgttatggcagaagcaggcggttccgtctttgcaaacatgccactgatttttgcgatcggtgtcgccctcggctttaccaataacgatggcgtatccgcgctggccgcagttgttgcctatggcatcatggttaaaaccatggccgtggttgcgccactggtactgcatttacctgctgaagaaatcgcctctaaacacctggcggatactggcgtactcggagggattatctccggtgcgatcgcagcgtacatgtttaaccgtttctaccgtattaagctgcctgagtatcttggcttctttgccggtaaacgctttgtgccgatcatttctggcctggctgccatctttactggcgttgtgctgtccttcatttggccgccgattggttctgcaatccagaccttctctcagtgggctgcttaccagaacccggtagttgcgtttggcatttacggtttcatcgaacgttgcctggtaccgtttggtctgcaccacatctggaacgtacctttccagatgcagattggtgaatacaccaacgcagcaggtcaggttttccacggcgacattccgcgttatatggcgggtgacccgactgcgggtaaactgtctggtggcttcctgttcaaaatgtacggtctgccagctgccgcaattgctatctggcactctgctaaaccagaaaaccgcgcgaaagtgggcggtattatgatctccgcggcgctgacctcgttcctgaccggtatcaccgagccgatcgagttctccttcatgttcgttgcgccgatcctgtacatcatccacgcgattctggcaggcctggcattcccaatctgtattcttctggggatgcgtgacggtacgtcgttctcgcacggtctgatcgacttcatcgttctgtctggtaacagcagcaaactgtggctgttcccgatcgtcggtatcggttatgcgattgtttactacaccatcttccgcgtgctgattaaagcactggatctgaaaacgccgggtcgtgaagacgcgactgaagatgcaaaagcgacaggtaccagcgaaatggcaccggctctggttgctgcatttggtggtaaagaaaacattactaacctcgacgcatgtattacccgtctgcgcgtcagcgttgctgatgtgtctaaagtggatcaggccggcctgaagaaactgggcgcagcgggcgtagtggttgctggttctggtgttcaggcgattttcggtactaaatccgataacctgaaaaccgagatggatgagtacatccgtaaccac

SEQ ID NO: 3 - protein, 699 aa, Bacillus subtilis
MFKALFGVLQKIGRALMLPVAILPAAGILLAIGNAMQNKDMIQVLHFLSNDNVQLVAGVMESAGQIVFDNLPLLFAVGVAIGLANGDGVAGIAAIIGYLVMNVSMSAVLLANGTIPSDSVERAKFFTENHPAYVNMLGIPTLATGVFGGIIVGVLAALLFNRFYTIELPQYLGFFAGKRFVPIVTSISALILGLIMLVIWPPIQHGLNAFSTGLVEANPTLAAFIFGVIERSLIPFGLHHIFYSPFWYEFFSYKSAAGEIIRGDQRIFMAQIKDGVQLTAGTFMTGKYPFMMFGLPAAALAIYHEAKPQNKKLVAGIMGSAALTSFLTGITEPLEFSFLFVAPVLFAIHCLFAGLSFMVMQLLNVKIGMTFSGGLIDYFLFGILPNRTAWWLVIPVGLGLAVIYYFGFRFAIRKFNLKTPGREDAAEETAAPGKTGEAGDLPYEILQAMGDQENIKHLDACITRLRVTVNDQKKVDKDRLKQLGASGVLEVGNNIQAIFGPRSDGLKTQMQDIIAGRKPRPEPKTSAQEEVGQQVEEVIAEPLQNEIGEEVFVSPITGEIHPITDVPDQVFSGKMMGDGFAILPSEGIVVSPVRGKILNVFPTKHAIGLQSDGGREILIHFGIDTVSLKGEGFTSFVSEGDRVEPGQKLLEVDLDAVKPNVPSLMTPIVFTNLAEGETVSIKASGSVNREQEDIVKIEK

SEQ ID NO: 4 - DNA, 2097 bp, Bacillus subtilis
atgtttaaagcattattcggcgttcttcaaaaaattgggcgtgcgcttatgcttccagttgcgatccttccggctgcgggtattttgcttgcgatcgggaatgcgatgcaaaataaggacatgattcaggtcctgcatttcttgagcaatgacaatgttcagcttgtagcaggtgtgatggaaagtgctgggcagattgttttcgataaccttccgcttcttttcgcagtaggtgtagccatcgggcttgccaatggtgatggagttgcagggattgcagcaattatcggttatcttgtaatgaatgtatccatgagtgcggttcttcttgcaaacggaaccattccttcggattcagttgaaagagccaagttctttacggaaaaccatcctgcatatgtaaacatgcttggtatacctaccttggcgacaggggtgttcggcggtattatcgtcggtgtgttagctgcattattgtttaacagattttacacaattgaactgccgcaataccttggtttctttgcgggtaaacgtttcgttccaattgttacgtcaatttctgcactgattctgggtcttattatgttagtgatctggcctccaatccagcatggattgaatgccttttcaacaggattagtggaagcgaatccaacccttgctgcatttatcttcggggtgattgaacgttcgcttatcccattcggattgcaccatattttctattcaccgttctggtatgaattcttcagctataagagtgcagcaggagaaatcatccgcggggatcagcgtatctttatggcgcagattaaagacggcgtacagttaacggcaggtacgttcatgacaggtaaatatccatttatgatgttcggtctgcctgctgcggcgcttgccatttatcatgaagcaaaaccgcaaaacaaaaaactcgttgcaggtattatgggttcagcggccttgacatctttcttaacggggatcacagagccattggaattttctttcttattcgttgctccagtcctgtttgcgattcactgtttgtttgcgggactttcattcatggtcatgcagctgttgaatgttaagattggtatgacattctccggcggtttaattgactacttcctattcggtattttaccaaaccggacggcatggtggcttgtcatccctgtcggcttagggttagcggtcatttactactttggattccgatttgccatccgcaaatttaatctgaaaacacctggacgcgaggatgctgcggaagaaacagcagcacctgggaaaacaggtgaagcaggagatcttccttatgagattctgcaggcaatgggtgaccaggaaaacatcaaacaccttgatgcttgtatcactcgtctgcgtgtgactgtaaacgatcagaaaaaggttgataaagaccgtctgaaacagcttggcgcttccggagtgctggaagtcggcaacaacattcaggctattttcggaccgcgttctgacgggttaaaaacacaaatgcaagacattattgcgggacgcaagcctagacctgagccgaaaacatctgctcaagaggaagtaggccagcaggttgaggaagtgattgcagaaccgctgcaaaatgaaatcggcgaggaagttttcgtttctccgattaccggggaaattcacccaattacggatgttcctgaccaagtcttctcagggaaaatgatgggtgacggttttgcgattctcccttctgaaggaattgtcgtatcaccggttcgcggaaaaattctcaatgtgttcccgacaaaacatgcgatcggcctgcaatccgacggcggaagagaaattttaatccactttggtattgataccgtcagcctgaagggcgaaggatttacgtctttcgtatcagaaggagaccgcgttgagcctggacaaaaacttcttgaagttgatctggatgcagtcaaaccgaatgtaccatctctcatgacaccgattgtatttacaaaccttgctgaaggagaaacagtcagcattaaagcaagcggttcagtcaacagagaacaagaagatattgtgaagattgaaaaa

SEQ ID NO: 5 - protein, 425 aa, Agrobacterium tumefaciens
MTAILENLAAARRAGKPAGITSVCSAHPVVLRAAIRRAAASQTAVLIEATCNQVNHLGGYTGMTPRDFVAFVNSIAAEEGLPAELLIFGGDHLGPNPWRREKAEDALTKAAAMVDAYVTAGFRKIHLDASMGCAGEPAALDDVTIAHRAAKLTAVAEKAATEAGLPKPLYILGTEVPVPGGADHVLETVAPTEPQAARNTIDLHREIFAQHGLSDAFERVIAFVVQPGVEFGSDNVVAYDPQAAQSLSAVLDGEPRLVFEAHSTDYQTEPALAALVRDGYPILKVGPGLTFAYREALYALDMIASEMVGTYGDRPLARTMEKLMLSAPGDWQGHYHGDDITLRLQRHYSYSDRIRYYWTRPEALAAVSTLHKALDGKTIPETLLRQYLGELPLAAVAGKEPEEVLVAAVDQVLATYHAATGEGRH

SEQ ID NO: 6 - DNA, 1275 bp, Agrobacterium tumefaciens
atgaccgccattttggaaaatctcgccgccgcgcgccgcgccggcaaacctgcgggcatcacttcggtctgctcggcccaccccgttgtcctgcgcgccgcaatccgccgcgccgccgccagtcaaacggccgtactgatcgaggccacctgcaatcaggtcaatcatctcggtggttataccggcatgacaccgcgtgacttcgttgccttcgtcaacagcatcgccgcggaagaaggactgcccgccgaactgctgatctttggcggcgatcatctcggccccaatccctggcgcagggagaaggccgaggacgcgctgacaaaagccgccgccatggtcgacgcctatgtcacagctggttttcgcaagatccaccttgatgcatcgatgggctgcgccggtgagccggcagccctggatgacgtcaccatcgcccaccgcgccgcgaaactcacagccgttgccgaaaaggcagccactgaggctggcctgccaaaaccgctttatattctgggcaccgaagtgccggtgcccggcggtgccgaccatgtgcttgagaccgtcgcaccgaccgaaccgcaggcggcgcgcaacaccatcgatcttcatcgcgaaatctttgcgcagcacggtctttccgatgcgttcgaacgggtcatcgcctttgtcgtgcagccgggtgtggaattcggcagcgacaatgtcgtcgcttatgatccgcaggcagcgcagagcctgagcgccgtgctggatggcgaaccgcgactggtcttcgaagcccattcgaccgattaccagaccgagcctgcccttgcggcactggtacgcgacggatatccgatcctcaaagttggaccgggcctcaccttcgcttaccgggaagcgctttatgcactcgacatgatcgcctccgaaatggtcggcacctatggcgaccgaccgctggcgcggactatggaaaaattgatgttaagcgcgccgggcgactggcagggccattaccatggcgacgacatcacgctccgattgcaacgccattacagctacagcgaccgcatccgttactactggacgcgaccggaagcgctcgcggccgtttccaccttgcataaggcactggatgggaagacaattcccgaaaccctgctgcgccaatatctcggcgaattgccgctcgcggcggttgcgggaaaggaaccggaggaggttctggtcgcggcggtggatcaggtgctggcgacctatcacgcggcgacgggcgaaggccgccac

SEQ ID NO: 7 - protein, 223 aa, Archaeoglobus fulgidus
MFKPKAIAVDIDGTLTDRKRALNCRAVEALRKVKIPVILATGNISCFARAAAKLIGVSDVVICENGGVVRFEYDGEDIVLGDKEKCVEAVRVLEKHYEVELLDFEYRKSEVCMRRSFDINEARKLIEGMGVKLVDSGFAYHIMDADVSKGKALKFVAERLGISSAEFAVIGDSENDIDMFRVAGFGIAVANADERLKEYADLVTPSPDGEGVVEALQFLGLLR

SEQ ID NO: 8 - DNA, 669 bp, Archaeoglobus fulgidus
atgttcaaaccaaaggccatcgcagttgacatagatggcaccctcaccgacagaaagagggctctgaactgcagggctgttgaagctctccgcaaggtaaaaattcccgtgattttggccactggtaacatatcttgttttgcgagggctgcagcaaagctgattggagtctcagacgtggtaatctgcgagaatgggggcgtggtgaggttcgagtacgatggggaggatattgttttaggagataaagagaaatgcgttgaggctgtgagggtgcttgagaaacactatgaggttgagctgctggacttcgaatacaggaagtcggaagtgtgcatgaggaggagctttgacatcaacgaggcgagaaagctcattgaggggatgggggttaagcttgtggattcaggctttgcctaccacattatggatgctgatgttagcaagggaaaagctttgaagttcgttgccgagaggcttggtatcagttcagcggagtttgcagttatcggcgactcagagaacgacatagacatgttcagagttgctggattcggaattgctgttgccaatgccgatgagaggctgaaggagtatgctgatttagttacgccatcaccagacggcgagggggttgttgaggctttgcagtttctgggattgttgcgg

SEQ ID NO: 9 - protein, 321 aa, Escherichia coli
MTKYALVGDVGGTNARLALCDIASGEISQAKTYSGLDYPSLEAVIRVYLEEHKVEVKDGCIAIACPITGDWVAMTNHTWAFSIAEMKKNLGFSHLEIINDFTAVSMAIPMLKKEHLIQFGGAEPVEGKPIAVYGAGTGLGVAHLVHVDKRWVSLPGEGGHVDFAPNSEEEAIILEILRAEIGHVSAERVLSGPGLVNLYRAIVKADNRLPENLKPKDITERALADSCTDCRRALSLFCVIMGRFGGNLALNLGTFGGVFIAGGIVPRFLEFFKASGFRAAFEDKGRFKEYVHDIPVYLIVHDNPGLLGSGAHLRQTLGHIL

SEQ ID NO: 10 - DNA, 963 bp, Escherichia coli
atgacaaagtatgcattagtcggtgatgtgggcggcaccaacgcacgtcttgctctgtgtgatattgccagtggtgaaatctcgcaggctaagacctattcagggcttgattaccccagcctcgaagcggtcattcgcgtttatcttgaagaacataaggtcgaggtgaaagacggctgtattgccatcgcttgcccaattaccggtgactgggtggcgatgaccaaccatacctgggcgttctcaattgccgaaatgaaaaagaatctcggttttagccatctggaaattattaacgattttaccgctgtatcgatggcgatcccgatgctgaaaaaagagcatctgattcagtttggtggcgcagaaccggtcgaaggtaagcctattgcggtttacggtgccggaacggggcttggggttgcgcatctggtccatgtcgataagcgttgggtaagcttgccaggcgaaggcggtcacgttgattttgcgccgaatagtgaagaagaggccattatcctcgaaatattgcgtgcggaaattggtcatgtttcggcggagcgcgtgctttctggccctgggctggtgaatttgtatcgcgcaattgtgaaagctgacaaccgcctgccagaaaatctcaagccaaaagatattaccgaacgcgcgctggctgacagctgcaccgattgccgccgcgcattgtcgctgttttgcgtcattatgggccgttttggcggcaatctggcgctcaatctcgggacatttggcggcgtgtttattgcgggcggtatcgtgccgcgcttccttgagttcttcaaagcctccggtttccgtgccgcatttgaagataaagggcgctttaaagaatatgtccatgatattccggtgtatctcatcgtccatgacaatccgggccttctcggttccggtgcacatttacgccagaccttaggtcacattctg

SEQ ID NO: 11 - protein, 321 aa, Bacillus subtilis
MDEIWFAGIDLGGTTIKLAFINQYGEIQHKWEVPTDKTGDTITVTIAKTIDSKLDELQKPKHIIKYIGMGAPGPVDMAAGVVYETVNLGWKNYALKNHLETETGIPAVIENDANIAALGEMWKGAGDGAKDVILVTLGTGVGGGIIANGEIVHGINGAGGEIGHICSIPEGGAPCNCGKTGCIETIASATGIVRIAKEKIANAKKTTRLKATEQLSARDVFEAAGENDEIALEVVDYVAKHLGLVLGNLASSLNPSKIVLGGGVSRAGELLRSKVEKTFRKCAFPRAAQAADISIAALGNDAGVIGGAWIAKNEWLKHQNC

SEQ ID NO: 12 - DNA, 963 bp, Bacillus subtilis
atggacgagatatggtttgcgggcattgacctgggaggaacgacgattaaactcgcttttattaatcaatatggcgaaattcagcataagtgggaagttccgacagataaaaccggcgacacgattactgtcacaattgcaaaaacaatcgacagcaagctggatgagctgcaaaaaccgaagcacatcatcaaatacatcggaatgggtgcaccaggccctgtagatatggcggcaggagtggtttatgaaacagtaaatctagggtggaaaaattatgctttgaaaaaccatctggagacagaaaccggcatcccagctgttatagaaaatgacgcgaatattgctgcgctcggggaaatgtggaagggagcgggtgatggcgcaaaagacgtcattctcgtgacgcttggcacaggagttggcggcggcatcattgcaaatggtgaaattgtacatggtataaatggcgccggcggagaaatcggccatatttgcagcatccctgaaggcggagcgccctgcaactgcggcaaaacgggctgtatcgaaacaattgcgtcagcaaccggaattgtaagaattgcaaaagaaaaaatagcaaatgctaaaaagacgacacgtttaaaagcaaccgaacaattgtcagcgcgagatgtgtttgaagcggcgggtgaaaatgatgaaattgcccttgaggtggttgattatgtagccaagcatcttggtttggtgctcggaaatttggcaagctcgcttaatccatccaaaatcgttcttggcggcggcgtatcgagagccggagaactgctgagatcaaaagtcgagaaaacattccgcaaatgcgcgtttccgcgggcagcccaagctgctgatatttcaatcgcagcacttggaaatgatgccggcgttatcggaggcgcttggatcgctaaaaatgaatggctgaaacatcaaaattgt

SEQ ID NO: 13 - protein, 549 aa, Escherichia coli
MKNINPTQTAAWQALQKHFDEMKDVTIADLFAKDGDRFSKFSATFDDQMLVDYSKNRITEETLAKLQDLAKECDLAGAIKSMFSGEKINRTENRAVLHVALRNRSNTPILVDGKDVMPEVNAVLEKMKTFSEAIISGEWKGYTGKAITDVVNIGIGGSDLGPYMVTEALRPYKNHLNMHFVSNVDGTHIAEVLKKVNPETTLFLVASKTFTTQETMTNAHSARDWFLKAAGDEKHVAKHFAALSTNAKAVGEFGIDTANMFEFWDWVGGRYSLWSAIGLSIVLSIGFDNFVELLSGAHAMDKHFSTTPAEKNLPVLLALIGIWYNNFFGAETEAILPYDQYMHRFAAYFQQGNMESNGKYVDRNGNVVDYQTGPIIWGEPGTNGQHAFYQLIHQGTKMVPCDFIAPAITHNPLSDHHQKLLSNFFAQTEALAFGKSREVVEQEYRDQGKDPATLDYVVPFKVFEGNRPTNSILLREITPFSLGALIALYEHKIFTQGVILNIFTFDQWGVELGKQLANRILPELKDDKEISSHDSSTNGLINRYKAWRG

SEQ ID NO: 14 - DNA, 1647 bp, Escherichia coli
atgaaaaacatcaatccaacgcagaccgctgcctggcaggcactacagaaacacttcgatgaaatgaaagacgttacgatcgccgatctttttgctaaagacggcgatcgtttttctaagttctccgcaaccttcgacgatcagatgctggtggattactccaaaaaccgcatcactgaagagacgctggcgaaattacaggatctggcgaaagagtgcgatctggcgggcgcgattaagtcgatgttctctggcgagaagatcaaccgcactgaaaaccgcgccgtgctgcacgtagcgctgcgtaaccgtagcaataccccgattttggttgatggcaaagacgtaatgccggaagtcaacgcggtgctggagaagatgaaaaccttctcagaagcgattatttccggtgagtggaaaggttataccggcaaagcaatcactgacgtagtgaacatcgggatcggcggttctgacctcggcccatacatggtgaccgaagctctgcgtccgtacaaaaaccacctgaacatgcactttgtttctaacgtcgatgggactcacatcgcggaagtgctgaaaaaagtaaacccggaaaccacgctgttcttggtagcatctaaaaccttcaccactcaggaaactatgaccaacgcccatagcgcgcgtgactggttcctgaaagcggcaggtgatgaaaaacacgttgcaaaacactttgcggcgctttccaccaatgccaaagccgttggcgagtttggtattgatactgccaacatgttcgagttctgggactgggttggcggccgttactctttgtggtcagcgattggcctgtcgattgttctctccatcggctttgataacttcgttgaactgctttccggcgcacacgcgatggacaagcatttctccaccacgcctgccgagaaaaacctgcctgtactgctggcgctgattggcatctggtacaacaatttctttggtgcggaaactgaagcgattctgccgtatgaccagtatatgcaccgtttcgcggcgtacttccagcagggcaatatggagtccaacggtaagtatgttgaccgtaacggtaacgttgtggattaccagactggcccgattatctggggtgaaccaggcactaacggtcagcacgcgttctaccagctgatccaccagggaaccaaaatggtaccgtgcgatttcatcgctccggctatcacccataacccgctctctgatcatcaccagaaactgctgtctaacttcttcgcccagaccgaagcgctggcgtttggtaaatcccgcgaagtggttgagcaggaatatcgtgatcagggtaaagatccggcaacgcttgactacgtggtgccgttcaaagtattcgaaggtaaccgcccgaccaactccatcctgctgcgtgaaatcactccgttcagcctgggtgcgttgattgcgctgtatgagcacaaaatctttactcagggcgtgatcctgaacatcttcaccttcgaccagtggggcgtggaactgggtaaacagctggcgaaccgtattctgccagagctgaaagatgataaagaaatcagcagccacgatagctcgaccaatggtctgattaaccgctataaagcgtggcgcggt

SEQ ID NO: 15 - protein, 450 aa, Bacillus subtilis
MTHVRFDYSKALTFFNEHELTYLRDFVKTAHHNIHEKTGAGSDFLGWVDLPEHYDKEEFARIKKSAEKIKSDSDVLLVVGIGGSYLGARAAIEALNHAFYNTLPKAKRGNPQVIFIGNNISSSYMRDVMDLLEDVDFSINVISKSGTTTEPAIAFRIFRKLLEEKYGKEEAKARIYATTDKERGALKTLSNEEGFESFVIPDDVGGRYSVLTAVGLLPIAVSGVNIDDMMKGALDASKDFATSELEDNPAYQYAVVRNVLYNKGKTIEMLINYEPALQYFAEWWKQLFGESEGKDEKGIYPSSANYSTDLHSLGQYVQEGRRDLFETVLNVEKPKHELTIEEADNDLDGLNYLAGKTVDFVNKKAFQGTMLAHTDGNVPNLIVNIPELNAYTFGYLVYFFEKACAMSGYLLGVNPFDQPGVEAYKVNMFALLGKPGFEEKKAELEKRLED

SEQ ID NO: 16 - DNA, 1350 bp, Bacillus subtilis
atgacgcatgtacgctttgactactcaaaagcgttgactttcttcaacgaacatgaacttacatacctgcgggactttgtaaaaacagcacaccataatatccatgagaaaacaggcgcgggcagcgattttctaggctgggtggacctccctgaacattatgataaagaagaattcgcgcgcatcaaaaaaagcgcggaaaaaatcaaatctgactctgatgtcttgcttgttgtcggcatcggcggttcttatcttggagcgcgggcagcgattgaagcgctgaatcacgcgttttataacactttgccaaaagcaaaacgcggcaatccgcaagtcatttttatcgggaacaacatcagttcatcttatatgagagacgtcatggatcttcttgaagatgttgacttctctattaatgtgatttctaaatcaggtacgacaactgaacctgcaatcgctttccgtattttccgcaagcttcttgaagagaaatacggtaaagaagaagcgaaagcgcggatttatgcaacaactgataaagagcgcggcgcattaaaaacgctttctaacgaagaaggctttgaatcattcgtaattcctgacgatgtcggcggccgttattcagttttaacagctgtaggtctcttgccgattgctgtcagcggcgtcaacattgacgacatgatgaaaggcgccctggatgcgagcaaagattttgcaacatctgaactggaagataacccagcataccaatatgcggttgttcgcaatgtcctttataataagggcaaaacaattgaaatgctcatcaactacgaaccggcgcttcaatactttgcggaatggtggaagcagctgttcggagaaagcgaagggaaagatgagaagggcatttatccttcttcagcgaactattcaacagaccttcattctttaggccagtatgtacaagaaggccgcagagatttattcgaaacggtcctgaacgtagagaagcctaaacatgaactgacaattgaggaagcggataacgatcttgacggcttgaactatttagccggtaaaactgttgatttcgttaacaaaaaagcattccaaggtacaatgcttgcccatacagacggaaatgttccgaacttaatcgttaacattcctgagctgaatgcatatacttttggataccttgtatatttcttcgaaaaagcctgcgcgatgagcggttacctccttggcgtcaatccgtttgaccagcctggtgtagaagcgtataaagtcaatatgtttgcgttactcggcaaacctggctttgaagagaaaaaagcagagcttgaaaaacgtctggaagat

SEQ ID NO: 17 - DNA, 1313 bp, Artificial Sequence
  Nucleotide sequence of SceI-tet-SceI fragment
tagggataacagggtaatatttacgttgacaccacctttcgcgtatggcatgatagcgcccggaagagagtcaattcagggtggtgaatatgaatagttcgacaaagatcgcattggtaattacgttactcgatgccatggggattggccttatcatgccagtcttgccaacgttattacgtgaatttattgcttcggaagatatcgctaaccactttggcgtattgcttgcactttatgcgttaatgcaggttatctttgctccttggcttggaaaaatgtctgaccgatttggtcggcgcccagtgctgttgttgtcattaataggcgcatcgctggattacttattgctggctttttcaagtgcgctttggatgctgtatttaggccgtttgctttcagggatcacaggagctactggggctgtcgcggcatcggtcattgccgataccacctcagcttctcaacgcgtgaagtggttcggttggttaggggcaagttttgggcttggtttaatagcggggcctattattggtggttttgcaggagagatttcaccgcatagtcccttttttatcgctgcgttgctaaatattgtcactttccttgtggttatgttttggttccgtgaaaccaaaaatacacgtgataatacagataccgaagtaggggttgagacgcaatcaaattcggtgtacatcactttatttaaaacgatgcccattttgttgattatttatttttcagcgcaattgataggccaaattcccgcaacggtgtgggtgctatttaccgaaaatcgttttggatggaatagcatgatggttggcttttcattagcgggtcttggtcttttacactcagtattccaagcctttgtggcaggaagaatagccactaaatggggcgaaaaaacggcagtactgctcgaatttattgcagatagtagtgcatttgcctttttagcgtttatatctgaaggttggttagatttccctgttttaattttattggctggtggtgggatcgctttacctgcattacagggagtgatgtctatccaaacaaagagtcatgagcaaggtgctttacagggattattggtgagccttaccaatgcaaccggtgttattggcccattactgtttactgttatttataatcattcactaccaatttgggatggctggatttggattattggtttagcgttttactgtattattatcctgctatcaatgaccttcatgttgacccctcaagctcaggggagtaaacaggagacaagtgcttagtagggataacagggtaat

SEQ ID NO: 18 - DNA, 90 bp, Artificial Sequence
  Primer sequence
caggagcactctcaattatgtttaagaatgcatttgctaacctgcaaaaggtcggtaaatcgctgtacggccccaaggtccaaacggtga

SEQ ID NO: 19 - DNA, 120 bp, Artificial Sequence
  Primer sequence
gccatctggctgccttagtctccccaacgtcttacggattagtggttacggatgtactcatccatcagcgatttaccgaccttttgcaggttagcttggcttcagggatgaggcgccatc

SEQ ID NO: 20 - DNA, 20 bp, Artificial Sequence
  Primer sequence
cgtcaaacaaattggcactg

SEQ ID NO: 21 - DNA, 20 bp, Artificial Sequence
  Primer sequence
gaacgtcaataacctgttcg

SEQ ID NO: 22 - DNA, 51 bp, Artificial Sequence
  Primer sequence
gtttaactttaataaggagatataccatgacaaagtatgcattagtcggtg

SEQ ID NO: 23 - DNA, 50 bp, Artificial Sequence
  Primer sequence
cgattactttctgttcgacttaagcattacagaatgtgacctaaggtctg

SEQ ID NO: 24 - DNA, 50 bp, Artificial Sequence
  Primer sequence
gttaagtataagaaggagatatacatatgaaaaacatcaatccaacgcag

SEQ ID NO: 25 - DNA, 50 bp, Artificial Sequence
  Primer sequence
tcagcggtggcagcagcctaggttaattaaccgcgccacgctttatagcg

SEQ ID NO: 26 - DNA, 50 bp, Artificial Sequence
  Primer sequence
cagaccttaggtcacattctgtaatgcttaagtcgaacagaaagtaatcg

SEQ ID NO: 27 - DNA, 51 bp, Artificial Sequence
  Primer sequence
caccgactaatgcatactttgtcatggtatatctccttattaaagttaaac

SEQ ID NO: 28 - DNA, 50 bp, Artificial Sequence
  Primer sequence
gctataaagcgtggcgcggttaattaacctaggctgctgccaccgctgag

SEQ ID NO: 29 - DNA, 50 bp, Artificial Sequence
  Primer sequence
ctgcgttggattgatgtttttcatatgtatatctccttcttatacttaac

SEQ ID NO: 30 - DNA, 90 bp, Artificial Sequence
  Primer sequence
cattccaaagttcagaggtagtcatgattaagaaaatcggtgtgttgacaagcggcggtgatgcgtacggccccaaggtccaaacggtga

SEQ ID NO: 31 - DNA, 120 bp, Artificial Sequence
  Primer sequence
gcctttttccgaaatcattaatacagttttttcgcgcagtccagccagtcacctttgaacggacgcgcatcaccgccgcttgtcaacacaccgatttggcttcagggatgaggcgccatc

SEQ ID NO: 32 - DNA, 20 bp, Artificial Sequence
  Primer sequence
catttggcctgacctgaatc

SEQ ID NO: 33 - DNA, 21 bp, Artificial Sequence
  Primer sequence
cgaacgccttatccggcctac

SEQ ID NO: 34 - DNA, 90 bp, Artificial Sequence
  Primer sequence
agactgtcatgaaaaagaccaaaattgtttgcaccatcggaccgaaaaccgaatctgaagagatgtacggccccaaggtccaaacggtga

SEQ ID NO: 35 - DNA, 120 bp, Artificial Sequence
  Primer sequence
caaaagcaatattacaggacgtgaacagatgcggtgttagtagtgccgctcggtaccagtgcacccatctcttcagattcggttttcggtccgatttggcttcagggatgaggcgccatc

SEQ ID NO: 36 - DNA, 20 bp, Artificial Sequence
  Primer sequence
aacttcggcaccagacgttg

SEQ ID NO: 37 - DNA, 20 bp, Artificial Sequence
  Primer sequence
tctgaacgtcagaagacagc

SEQ ID NO: 38 - DNA, 90 bp, Artificial Sequence
  Primer sequence
aaacgttgcagacaaaggacaaagcaatggcaatccacaatcgtgcaggccaacctgcacaacagtacggccccaaggtccaaacggtga

SEQ ID NO: 39 - DNA, 119 bp, Artificial Sequence
  Primer sequence
gtgtttacgcgtttttcagaacttcgctaacaatctcaaccgcttctttctcaatctgcttgcgctgttgtgcaggttggcctgcacgattgtgttggcttcagggatgaggcgccatc

SEQ ID NO: 40 - DNA, 23 bp, Artificial Sequence
  Primer sequence
cggtcaaaacgattaaagacaag

SEQ ID NO: 41 - DNA, 20 bp, Artificial Sequence
  Primer sequence
ccagtcgccagctaatgatg

SEQ ID NO: 42 - DNA, 90 bp, Artificial Sequence
  Primer sequence
gttaacttaaggagaatgacatggcggtaacgcaaacagcccaggcctgtgacctggtcattttctacggccccaaggtccaaacggtga

SEQ ID NO: 43 - DNA, 120 bp, Artificial Sequence
  Primer sequence
aagcgcagatattactcaaactcattccaggaacgaccatcacgggtaatcatcgccaccgaggcgaaaatgaccaggtcacaggcctgggctgtttggcttcagggatgaggcgccatc

SEQ ID NO: 44 - DNA, 21 bp, Artificial Sequence
  Primer sequence
gatttgctcaaatgttccagc

SEQ ID NO: 45 - DNA, 20 bp, Artificial Sequence
  Primer sequence
gcaacatgcttttcaaagag

SEQ ID NO: 46 - DNA, 54 bp, Artificial Sequence
  Primer sequence
gttaagtataagaaggagatatacatatgaacaccgaacatccgctgaaaaatg

SEQ ID NO: 47 - DNA, 50 bp, Artificial Sequence
  Primer sequence
cggtggcagcagcctaggttaattactcgagaatcagtttgaattcaccg

SEQ ID NO: 48 - DNA, 50 bp, Artificial Sequence
  Primer sequence
gtttaactttaagaaggagatataccatgttcaagccgaaagcgatcgcg

SEQ ID NO: 49 - DNA, 52 bp, Artificial Sequence
  Primer sequence
gattactttctgttcgacttaagcattaacgcagcaggcccagaaactgcag

SEQ ID NO: 50 - DNA, 54 bp, Artificial Sequence
  Primer sequence
catttttcagcggatgttcggtgttcatatgtatatctccttcttatacttaac

SEQ ID NO: 51 - DNA, 50 bp, Artificial Sequence
  Primer sequence
cggtgaattcaaactgattctcgagtaattaacctaggctgctgccaccg

SEQ ID NO: 52 - DNA, 52 bp, Artificial Sequence
  Primer sequence
ctgcagtttctgggcctgctgcgttaatgcttaagtcgaacagaaagtaatc

SEQ ID NO: 53 - DNA, 50 bp, Artificial Sequence
  Primer sequence
cgcgatcgctttcggcttgaacatggtatatctccttcttaaagttaaac

SEQ ID NO: 54 - protein, 219 aa, Archaeoglobus profundus
MFKALVVDIDGTLTDKKRAINCRAVEALRKLKIPVVLATGNISCFARAVAKIIGVSDIVIAENGGVVRFSYDGEDIVLGDRSKCLRALETLRKRFKVELLDNEYRKSEVCMRRNFPIEEARKILPKDVRIVDTGFAYHIIDANVSKGKALMFIADKLGLDVKDFIAIGDSENDIEMLEVAGFGVAVANADEKLKEVADLVTSKPNGDGVVEALEFLGLI

SEQ ID NO: 55 - DNA, 657 bp, Archaeoglobus profundus
gtgttcaaggctttggtagttgatatagacggaactttgacggataagaagagggcaataaactgcagagcggtcgaagcacttagaaaactaaagattcctgttgtcttggcaaccggaaacatttcatgctttgcaagggctgtagctaagattataggtgtttccgatattgtaatagctgagaacggaggtgttgtcagattcagctacgacggagaggacatagttctgggggatagaagtaaatgcttaagagctttggagacacttagaaaacgcttcaaagtagagcttctcgacaacgaatataggaagtctgaggtctgcatgaggaggaacttccctatagaggaagctagaaagatactgccaaaagatgttagaatagtcgatacaggcttcgcataccacataatcgatgcaaatgtcagcaaggggaaggctttgatgttcatagccgataagcttggcttggacgttaaggatttcattgcgataggtgattccgaaaacgacattgaaatgttggaagttgcaggttttggcgttgcagttgcgaatgcggatgaaaagcttaaggaggtagcggatttggtcacatcgaagcctaatggagacggagttgtcgaagctcttgagttcttgggactcatt